European Patent Application EP 4 389 896 A1, published June 26, 2024. Title: 一种诱导单倍体的方法及其在植物育种中的应用. Applicant: 中国水稻研究所. Application CN. The sequence listing filed with the application follows.

SEQUENCE LISTING (7 sequences)

SEQ ID NO: 1 - DNA, 6654 bp, (Oryza sativa)
  misc_feature 1..6654: note = OsCPRO1 (LOC_Os03g47740)
  source 1..6654: mol_type = genomic DNA
ggtttaaaccccccaaaccccacccaataatcctcctccttaatgataaacacgaagaaaattaaatactccctcccacaatttttcctttttctttctttcttttggaggccctccacaattattttattttggttgttggtggtagtggatggtgtttcttttttattccatttgtttatttatttttggcaacaacaagaagaagaggagagagagaagtagaagaagagaggagagaagctcctctctctctctcttgccttttttttttcttctctttttcatattgttatcttgggatctgatttttgtccccatactgggagggaaagaggagaggagggattgattttctttctcctcctcttcttgttcttcttcttgttgttccactcttattgttcatcatcctcctcctcatagctgaccaaatctctgctgtgacagcaatctctgctgcttggttctgcctcccatgaggagcacaccatcaggtctcccttccatcttgctcgaattttttatcaccccatctgcatcatttggtctctgttggttgcagcagaagaaaaaatctatttttttttgtgtgcatattcctcccccgaggacacgtgatttgctcttcttcttgctttgctttgcttctggatttgtgttgtctgattttggtgggtgcaactaatcctttttgttattcccgcgaggggtggtgttgtcatgagctcaatcattgggttggtctctgtctctctgagagtctgaattatgtgtgcacgggacggggtttgctttgctttctttgatagcggtggagcttagcgtctctggatgaattgcgaggttttcttggtgtttctgcgtgtttaattgacttggggatctgtaattcttgaggctccgtctcaggaattttgtgtttctttgggttggttcatggatgaactgaaggtatggtgttttctgcagttttagttggtgtttcctttttacatcctcacctcaaaagttgttctctggtggtgtggatgcttggaggaactgagcttggtttgctggcttcagaatccatggcttgtgttcttgaattctgggtttttgtggcgttcttggtggctcaaccaccatttggtgttgggagaagagctctgagtttctagcagctgcttctccagctaccggtagagctggcttttttttgggagagatgacagaattgagcttgattacagtggagtcctactttgatttgtggcttgtgttcttgaatctttaatctctgtggatgcctgcatgaaagccatatgctcataaaaagccctgttcctttttctcttttctgttgtggaaatgattcttgtgttggattgctatctcatattcctcttgtaatcgaattcttagctctcttctcatcagaatttgggtgtgcctcgtattctgttgtgcgtggcaacaaagtttttgccttggtcatttctcctagtttccacctctttcatatcgttaaaaacaagtggaaaatttgagatgtaaacaagtaaaaaaaaagaagtaacttttattttctctttgctggtctctattctctagttagtcatctcaggtcattttatctcgtctttcagtgtgattacaaagcaaggaaccctcctaccgcgtcgctgagctgatgaaggagctctgacgactcggatgcattcttctgccatcaatcaattgatccaacaaggtattgaaatagtattccatttataagttctttctttttctcaagaaaaaaaaaccctacaattttatctgtggccttgcagttcttgtatgtggtatagaaccacttatctcattgggttcttgaaaggtcgcctaatcttgatgaaataggaagaatttatagccacattctcgccgtcttgattatcttgataaggaaggagcaaaaggccaataacctagctataaactcagatgaaggaccacctgaagttctgtacctttagccagcaaactggcatcttaccttgtcacttcatagtttatattctcttgtttcttgagcatataacctgtgttcttccctacaaatatagtaagaaagaaaagaacaaaacagaggtggtaactgctgccaaagctgtgggtctgagcctcactcactcgtgactggcctttgtgtgtatcttgtgtccttgcaatagtaacagaaccgtacttgctttcccaaaaaaaaaaaagaaagaaagatctggtgattatagtgtgttttgtttcttcttaactatttcattatgtggtgtagaatttgattgtctcatatataattcctaactgtacctttttgttgtcattgttttgttgaacctttttccttccccctttgacaggcaactcgatcggaatttgagtttggtgaactctgtaattgattccctgcaagtatccatgcctttgcagcaatcttgctaattgagttgtcaaagctgcatacatggctacttactactcgagccctggcaatgaaagggactcgcaagctatgtacccagcggattcaggcaattcatcatatcctgtgccatcagcaataggaaacatgttatatcctggcaatgggtcttctgggccatacacggaattcagtggcattatccagcatcagcagaatttcatggagctgcctggccatccaactgcgatctctcaagattcatcgtcacgggaacctaacatggtcgcgtcgtacatggatcagcgctcttttggacctgccaaagatatgagaaatgagatgttgatgcatctgatggatggagcacataatgctggtgctgatctcatccacaatgacactcatagcagcgcgcagattgagtttggcctattgaacaaccacaattcgatgagcgttgcaccagcaccaggccaaggattgtctctgagcctcaacacgcatatcctggcgccttcgtatccatactggtctgcgaaaacagagttgctaacaccacactcttaccatggtgatgacaacagaatgaagaatatgcaatctgaggcctcacaggcaatcagaaactcaaagtatctgaaagcagcacaagaattgcttgatgaggtcgtcagtgtttggaagagtataaagcagaaggctcagaaagaccaggctgaagcaggaaaatcagataacaaagaagccgaggggggttcgaaaggtgagggggtatcttccaacccacaggagtctactgccaatgctgcaccagagatttctgctgctgagaaacaagagctccagaataagatggcaaaacttatggccatgttggatgaggtgtgtgaatttgttgcccttctatttcttaaaacaaaaattatattgcccttccctatacctcgctatgaaatcgaagtgtcataatggtttgtttgtgcttggctaaattcataccaataatttgcacaaagattactaatatgagcaggcttaatccagatactccaaagtaaagctccagaaacaaatacttgtctagtagcagttgcagcttattctctcgtgtgccaaaagtcaattgcgttgtcctgccttccgttgtcttcctagaaaagtattggttggacactggaatctccaccaaatcagtgttagatatgaccttagtattcactattagcatagatgggtcatgatccacagttcagaactgttttgacttattgctaaaagaaatgttttggcttctaacaagaacttcataagttgggcttcttacagaagttagagagatgggtcaaagcctcgaaggtaactagtctaggtgggtttagaaagcttagctgcctatagtcttacatgggaaaagcctttatcttctaaatgctcaagtttttatcttaaggccctccaaacaagtttgagaaagtcacatgttctattgaagtgtccagtagctgcaggaactaaaaataaaaatctctttcgagaagtcaaactgatagcattatcaataagatgagtagtggttttactggcaagctaatgatatccttgctggtttgtaatcataccatttgttttaattttcaggtggaccgaaagtacaaacactattatcatcaaatgcaaattgtagtctcatcttttgatatggttgctgggtctggagctgccaagccttatactgcagtggcccttcagacaatctcaaaacatttcagatgtctgaaagatgctatcaacgatcagatcaatgttatccggaagaaacttggagaggaggagagttcatctggcaaagagggaaaattaacgcgcctccgttatattgaccagcaattaagacaacagcgcgctttccagcagtatggtttgttacagcaaaatgcttggaggccacagaggggactgcccgaaaactcagtttcaattcttcgtgcttggctttttgaacacttccttcacccgtaagtgactttctttatacactcattttcatttgcctgttttttcttttgttgtcatgacattttgttgctttcttaggtatccaaaagattcagaaaagctgatgctagcgagacaaactggcttaacaagaagtcaggtattttttttcctatcatacaaagacaacctgttatcttatcataataacataccccatccgtcccaaaaaaaagtccaatcctaactacgaacctggatacatgtgtgtccagatttgtagctagaatttgcttcttttttttgggacaaagtagtagttagcaatcattgggatgtgtttatctagttaaaatagatggccacgtgttggtattgctaatgcatccggatgtatacccatgtgctgcaaaatctctgccatgatactgggcaactgtttattatttgcatgcacatcggcctttttctcagaataggtctgaaatctattaaaccctgtttcatcagttctggaatcatactatgttgtaacgctggatgctaatacaattttggatttgaatgggtacaaatgtttgtaaattacctttctttttgcagaactttgcactctgcatcaattcattggatagaattagtttgctgaactcaccaatattcttctttgtcctagatttcaaattggttcataaatgcccgtgtccgcctgtggaaaccgatgatcgaagacatgtataaagaagagattggggaggcggatctcgactcgaactcctcctccgacaacgtaccaaggagcaaggacaaaatagcaacatctgaagataaggaagatctgaaaagctctatgagccagacttatcaaccaagccaattaggtgaatccaaagccaacatcgggatgatgagccttggtggggcaccagccggcttccacaacgaaggcaaccaggatgacagcttcatgaacctaatgctgaaggaccaaaggccgggcgaagccgaaggcagcctcctccatgatgccgtcgcccatcattccgatgagaacgctcggttcatggcttaccatttgtcggggctcggaagatacgggaacagcaatgtgtcattgacacttggcttacagcatcctgacaacaggctttcggtacagaacactcatcagccaggtttcgccggtgctggagaagaaatttacaactccaccgcttctctcggtgtcgctgcagcttcctcttcggactacgaatccacgaaccaaatagatcaaaggcaacggttcgaaccatcgcctctaatgcatgattttgtggcctaagatgctcaaaataccaaaaatatatggaggcaagatttgcctggggggagcatttgtaatttgtagtgccagaataacatgcctcagaaagcatggaaattgttagctgtagttgcatttggtacagaagaggggggtatagcatgaaatgtaatataattaagtttagcaggtgggggtttatagggggtaaagaatcctgtaaaaatggaatacatcatacatgtaaaagattatgattttcagaaccattctgtaaaaaaaaacacacctgtaatgactacttatcatccaggtatatgttgttcagcctattgacaaaataaaaaaagaaagaaagccagaaaagaaaagatcgaagatcaatggacagatcgctggggaatcttcagctttctgttctgcatctgcaagttgatgcttcaggctttatgttactggagttgagcaccagctgttgctctctcctcttttatctctgtggagatggtttaatttgtcggtccatgcactgtttgccatttcatctcatttcatttccattacaatttaaaattctaattggcagcccttgccggtgcaggagcagctgcaggattgaagctgcagtgtggctgccccaggcccagggactgggctcatgcattttttttgtacgagtaaatgcgccctgttgctgtcatgtgggcccgggaactatggcttctctgtgggttcgatgaccccaaacccaaaggcttttaacaaccaccacttgtcaattattgaggaaccggctgagctggctttgtgaattgttaaggcgacctcacctcctgcagttaggactttgatcattgtggtttgtttaaattgtatatatggttggttggtatggattgag

SEQ ID NO: 2 - DNA, 2028 bp, (Oryza sativa)
  misc_feature 1..2028: note = OsCPRO1 (LOC_Os03g47740)CDS
  source 1..2028: mol_type = genomic DNA
atggctacttactactcgagccctggcaatgaaagggactcgcaagctatgtacccagcggattcaggcaattcatcatatcctgtgccatcagcaataggaaacatgttatatcctggcaatgggtcttctgggccatacacggaattcagtggcattatccagcatcagcagaatttcatggagctgcctggccatccaactgcgatctctcaagattcatcgtcacgggaacctaacatggtcgcgtcgtacatggatcagcgctcttttggacctgccaaagatatgagaaatgagatgttgatgcatctgatggatggagcacataatgctggtgctgatctcatccacaatgacactcatagcagcgcgcagattgagtttggcctattgaacaaccacaattcgatgagcgttgcaccagcaccaggccaaggattgtctctgagcctcaacacgcatatcctggcgccttcgtatccatactggtctgcgaaaacagagttgctaacaccacactcttaccatggtgatgacaacagaatgaagaatatgcaatctgaggcctcacaggcaatcagaaactcaaagtatctgaaagcagcacaagaattgcttgatgaggtcgtcagtgtttggaagagtataaagcagaaggctcagaaagaccaggctgaagcaggaaaatcagataacaaagaagccgaggggggttcgaaaggtgagggggtatcttccaacccacaggagtctactgccaatgctgcaccagagatttctgctgctgagaaacaagagctccagaataagatggcaaaacttatggccatgttggatgaggtggaccgaaagtacaaacactattatcatcaaatgcaaattgtagtctcatcttttgatatggttgctgggtctggagctgccaagccttatactgcagtggcccttcagacaatctcaaaacatttcagatgtctgaaagatgctatcaacgatcagatcaatgttatccggaagaaacttggagaggaggagagttcatctggcaaagagggaaaattaacgcgcctccgttatattgaccagcaattaagacaacagcgcgctttccagcagtatggtttgttacagcaaaatgcttggaggccacagaggggactgcccgaaaactcagtttcaattcttcgtgcttggctttttgaacacttccttcacccgtatccaaaagattcagaaaagctgatgctagcgagacaaactggcttaacaagaagtcagatttcaaattggttcataaatgcccgtgtccgcctgtggaaaccgatgatcgaagacatgtataaagaagagattggggaggcggatctcgactcgaactcctcctccgacaacgtaccaaggagcaaggacaaaatagcaacatctgaagataaggaagatctgaaaagctctatgagccagacttatcaaccaagccaattaggtgaatccaaagccaacatcgggatgatgagccttggtggggcaccagccggcttccacaacgaaggcaaccaggatgacagcttcatgaacctaatgctgaaggaccaaaggccgggcgaagccgaaggcagcctcctccatgatgccgtcgcccatcattccgatgagaacgctcggttcatggcttaccatttgtcggggctcggaagatacgggaacagcaatgtgtcattgacacttggcttacagcatcctgacaacaggctttcggtacagaacactcatcagccaggtttcgccggtgctggagaagaaatttacaactccaccgcttctctcggtgtcgctgcagcttcctcttcggactacgaatccacgaaccaaatagatcaaaggcaacggagcagctgcaggattgaagctgcagtgtggctgccccaggcccagggactgggctcatgcattttttttgtacgagtaaatgcgccctgttgctgtcatgtgggcccgggaactatggcttctctgtgggttcgatga

SEQ ID NO: 3 - protein, 675 aa, (Oryza sativa)
  REGION 1..675: note = OsCPRO1 (LOC_Os03g47740)
MATYYSSPGNERDSQAMYPADSGNSSYPVPSAIGNMLYPGNGSSGPYTEFSGIIQHQQNFMELPGHPTAISQDSSSREPNMVASYMDQRSFGPAKDMRNEMLMHLMDGAHNAGADLIHNDTHSSAQIEFGLLNNHNSMSVAPAPGQGLSLSLNTHILAPSYPYWSAKTELLTPHSYHGDDNRMKNMQSEASQAIRNSKYLKAAQELLDEVVSVWKSIKQKAQKDQAEAGKSDNKEAEGGSKGEGVSSNPQESTANAAPEISAAEKQELQNKMAKLMAMLDEVDRKYKHYYHQMQIVVSSFDMVAGSGAAKPYTAVALQTISKHFRCLKDAINDQINVIRKKLGEEESSSGKEGKLTRLRYIDQQLRQQRAFQQYGLLQQNAWRPQRGLPENSVSILRAWLFEHFLHPYPKDSEKLMLARQTGLTRSQISNWFINARVRLWKPMIEDMYKEEIGEADLDSNSSSDNVPRSKDKIATSEDKEDLKSSMSQTYQPSQLGESKANIGMMSLGGAPAGFHNEGNQDDSFMNLMLKDQRPGEAEGSLLHDAVAHHSDENARFMAYHLSGLGRYGNSNVSLTLGLQHPDNRLSVQNTHQPGFAGAGEEIYNSTASLGVAAASSSDYESTNQIDQRQRSSCRIEAAVWLPQAQGLGSCIFFVRVNAPCCCHVGPGTMASLWVR

SEQ ID NO: 4 - DNA, 5254 bp, (Oryza sativa)
  misc_feature 1..5254: note = OsCPRO2 (LOC_Os12g43950)
  source 1..5254: mol_type = genomic DNA
gtggtggttacaccagcaaataactccaagcagcagcatcagcagcagcagcaacagttgagaggaggaggaggaggaggttagctagctcgtcagtataatccttctcgacagcaactaataaaggaacaagcaaaactatttctttaggaggcaaacattattccatatttggtgctgctgttagtgggtggtctgagctttttttatttaggcaacaaggagcaagctagcacaactgctgcttgctagagagaggagagaagaaggaggagaagaagaggagagagaggagctctgagctctgtgctctctcttgctgctgctgctggctgctgctcacttttccttttgggattgttacttattttaatcctgggatctgattttgtccccatattgggaggatcgattatctttctcccctcctctcctctcctctcatcccctctcccctatctatctgtcttgaagaagatcagctggctgctttggtgtcaatcgctgctgcagttcctgttgcctttgccctgcgccccatcaggagcacaccctcaggtctctcctccattttcttattgccttctcttgtaccatctgctcctcctcctcctccttattgcagcatcatcagcaacggattgcatgcatgacctctgttcttggttcttggcttcagttcgatgatggtggaatttcactgaattatggtgtgtttcttgctcttgtggttggtgcttaacgctggctctcttgggtttctgagctcttcttgccttgttgggttagagagctagggtactgctcttcccttccatctgaatttttcagcttcttttgatgtttggggatttttttttgcttgctgctggtttttctcgatgaaccgaaagctcaggtgcaaagattgtttcttttgactgaccttgaggttccatgccctcaacctcaacaaagttcttgcctttctttggtgtatagattcttgtggagaaattcttgtgttcaaaactcatatgcttagttttctccgaattatgagttcttgttttcttctcggattgtaaagcaacccacttttttgtggctttgcccataatttgagcttatgtacgaacaggctttgcgattgccgactaaattgtcctagctttctttcttttttttccctttcttcctcgacgtttacatggaagcagtcttcaaaaaatgttttcatggaagctgggctctcaaaagccaaatttcctgttacttttacctttttgcagtagttcttctgttgagttactgcactccagacactttatgctaaggaaatcttgcttgtttttcatcaaaatcttgtgcttctttgttctgtatgtaggttatacatgtgccttggagttttctctttggctctactctctaaaaatctagctatgaaaaagaatttgtttagactgacaaacaggctgctaagtaagttcatctcttgcagattttgattggtagctgtgttcgtagcaataacagcctggcagagaatctttgagaagttgcagtctattagttcaacaaggtactcatcatgataaatgatcattactcactcaagagtcatatgttcaaaccttatctatccaatgcaattctccttttcatgatactactgtggtttccccatgttgcttttatgaaaagaaaagaaaacactgggcagtcatttgattttggtttatggtgttgtccggttgtttatcttggtatataacaagaggaattcacaagtagatattcttataacatcttgttagcaaaggaggaccacaaagtccaaaacttttttgatccaatcttaaaaatggaggaccacttgtggctttagcctgcaaatcggcatgtcacattgtcagttcatatattatcgcacttctcgagcaaagttttgcaggtgactgcatttctatcagatagaatcctgccaaaacttagcctgagccccaattctgattactcacttatgactggcattctttgtgtgcttctgctgtatctatattaacagtttgctcaattaaactttcttgtctttgtttgtgcaaagtgttttgaagttttccattgaactgctttacaagcacttgcctgcagttatttttgttggcattggtgtgctgttattttacaatctcagaggagagaactccttattcaatatttgaacttccttgggggtgtcttatcagtccatttcatgtactcaattgcagggaagttgaacgggatcaagtttagtctggataacaaaatattgatgtcctgctggaatcatcaatcaagtcaacgtcaaagctggttcttcatatacatatatgcttttgcagtaatctcgagcaataagtagttataattgcgagatggctacttactattcaagccctggtagcgaaagagactcgcagaccatgtactcaagagacccaggcagtgcatcctatcctatgtcatcagctctagggaacttgctctatctgaacaatccatcttctggaccttatacggagttcagcggcattctgcagcctcagcagaattgcatggagatgcctggccctgggcatgcgtcagcaatgtcacaagacccctcttcaagggagtccgacatgctttcttcgcaccagggtcaacgctctttcagccatgtcaaagatatgaaaaatgagatgttgatgcatatgatggatggagcacaaggtagtggctctgagctcatccatgatgatgcccacactggttcacagcttgagtttggtgttctgaataatcacaactcatcaagtgttccatcaatgcaaagccaagggctatctctgagcttgaacacacaaatcatggcgccttccttaccgtactggtctataaagccagacatgttaacgccgcagtcttaccatgacaaccttagaggggaagacatgcggatgaagaatttgcagtccgaagcttcacgcgcaatccggaactcaaggtatctcaaggcagcacaagaactgcttgatgaggtcgtgagtgtttggaagagcataaaacaaaaggctcagaaagagaaggttgaatcaggaaaagcagatggcaaagagactgatggagggccaaaaagtgagggtgtatcttctaatccacaagaatctggcgctaatgcagcacctgagctttccactgctgagaagcaagagcttcagaacaaaatggcaaaactgatggcaatgttggatgaggtgagtactctaggagtctattgttttgtacttctctttctttttaaacagaagtgcaaccccaatttctttgagttgagattacagtatcaatagttttataggactgatccttggtatatgtatacaagagtagatatacagtttacttatagcacagtaatcttagttaattgattggcaaatcattttaactcaaaaaaatatatatttcaggtggaccggaaatacaagcattattaccaccaaatgcaaaccgtggtttcatcgtttgatgtggtagctggaccaggatctgcgaagccttacacagcagttgctcttcagacaatctcacggcactttcggtgcctgaaggatgctatcaatgatcagatcaatgttatcaggaaaaagcttggcgaggaagagaactcatctggcaaggagggaaaattaacccgcctccggtacattgatcagcagctaaggcaacaacgtgctttccaacagtacggtatgattccacaaaacgcctggagaccacagaggggactgcctgaaaactctgttacaattcttcgcgcttggctgtttgaacacttcctccatccgtaagtttcatcctttatgctgttctttccagcattccctcttttcttttctcttatcatcctccacaacaattttgcaggtacccaaaagattccgagaagttaatgcttgctaggcagactggcctgactaggagtcaggtaaatattgtttatcttttttgtgcactggaccattgatccacatttgatgttttaacttcttatcctagaagcattttgtgtttcttcaagagttcaacatgttgactgcttcatgcttctcctgttctccagatttcgaattggttcataaatgcccgtgtccgcctttggaaaccaatgattgaagacatgtacaaagaagagattggtgatttagagcaagactccaactcttcctctgacaatgcaccaagaagtaaggataaaatggcatcttcagaagacaaggaggatctcaaaaactccagggcacggatttgcgaaacaagccaattgagcgagtcgagaaccagcattggagcaatgaatgttggcggagcgcctgttggcttccagaatgagcccaatcctgatgacagtttcatgaacctgatgctgaaggaccagcgatcgaacgaagtggatggcggcctccttctccacaacactgtcgcgcagcactcagacgagaacgcccggttcatggcctatcacttggcagagcttgggagatacggcaatggcaatgtgtcgctgacactgggcttgcagcactccagcagcaacctcgttcctaatgctcagccaggtttccctggtgttaatgaggatgacatctacaatgctactgctcctcttggtgtcaccgtcgcatcttcggactatgattcgatgaatcagatggatcaacggcaacggtttgagcattcacctcttctgcatgattttgtggcctgaagacagcagagaaacaatcaggaccatggacattaagagagagaattggggggcagcatttgtaacacctagtgggagaataacatgcctgaaagggcatgggatttgtagctttgtagttgccatttaatacagaagaggaggtatagcaggaaatgtaatataaggttagatggtgggggtgatagggtaaagaatcatatgtaaagataaaatccatcattactatatatatatacgtgtaaaagcttgtgatttgagcaccatattgtaaagtaatggttacttagggctgtccaattatacactctcacactactattagagcttttctgtcattcttttacacgtgtaagtggagctgaaaacttgctgtgtccagcaagttatgcagatttgcgttaagttctgttgtttttgttgtggagcactacagctcagctgggtgaaaataaacttgagttcatgttcatgtca

SEQ ID NO: 5 - DNA, 1944 bp, (Oryza sativa)
  misc_feature 1..1944: note = OsCPRO2 (LOC_Os12g43950)CDS
  source 1..1944: mol_type = genomic DNA
atggctacttactattcaagccctggtagcgaaagagactcgcagaccatgtactcaagagacccaggcagtgcatcctatcctatgtcatcagctctagggaacttgctctatctgaacaatccatcttctggaccttatacggagttcagcggcattctgcagcctcagcagaattgcatggagatgcctggccctgggcatgcgtcagcaatgtcacaagacccctcttcaagggagtccgacatgctttcttcgcaccagggtcaacgctctttcagccatgtcaaagatatgaaaaatgagatgttgatgcatatgatggatggagcacaaggtagtggctctgagctcatccatgatgatgcccacactggttcacagcttgagtttggtgttctgaataatcacaactcatcaagtgttccatcaatgcaaagccaagggctatctctgagcttgaacacacaaatcatggcgccttccttaccgtactggtctataaagccagacatgttaacgccgcagtcttaccatgacaaccttagaggggaagacatgcggatgaagaatttgcagtccgaagcttcacgcgcaatccggaactcaaggtatctcaaggcagcacaagaactgcttgatgaggtcgtgagtgtttggaagagcataaaacaaaaggctcagaaagagaaggttgaatcaggaaaagcagatggcaaagagactgatggagggccaaaaagtgagggtgtatcttctaatccacaagaatctggcgctaatgcagcacctgagctttccactgctgagaagcaagagcttcagaacaaaatggcaaaactgatggcaatgttggatgaggtggaccggaaatacaagcattattaccaccaaatgcaaaccgtggtttcatcgtttgatgtggtagctggaccaggatctgcgaagccttacacagcagttgctcttcagacaatctcacggcactttcggtgcctgaaggatgctatcaatgatcagatcaatgttatcaggaaaaagcttggcgaggaagagaactcatctggcaaggagggaaaattaacccgcctccggtacattgatcagcagctaaggcaacaacgtgctttccaacagtacggtatgattccacaaaacgcctggagaccacagaggggactgcctgaaaactctgttacaattcttcgcgcttggctgtttgaacacttcctccatccgtacccaaaagattccgagaagttaatgcttgctaggcagactggcctgactaggagtcagatttcgaattggttcataaatgcccgtgtccgcctttggaaaccaatgattgaagacatgtacaaagaagagattggtgatttagagcaagactccaactcttcctctgacaatgcaccaagaagtaaggataaaatggcatcttcagaagacaaggaggatctcaaaaactccagggcacggatttgcgaaacaagccaattgagcgagtcgagaaccagcattggagcaatgaatgttggcggagcgcctgttggcttccagaatgagcccaatcctgatgacagtttcatgaacctgatgctgaaggaccagcgatcgaacgaagtggatggcggcctccttctccacaacactgtcgcgcagcactcagacgagaacgcccggttcatggcctatcacttggcagagcttgggagatacggcaatggcaatgtgtcgctgacactgggcttgcagcactccagcagcaacctcgttcctaatgctcagccaggtttccctggtgttaatgaggatgacatctacaatgctactgctcctcttggtgtcaccgtcgcatcttcggactatgattcgatgaatcagatggatcaacggcaacggtttgagcattcacctcttctgcatgattttgtggcctga

SEQ ID NO: 6 - protein, 647 aa, (Oryza sativa)
  REGION 1..647: note = OsCPRO2 (LOC_Os12g43950)
MATYYSSPGSERDSQTMYSRDPGSASYPMSSALGNLLYLNNPSSGPYTEFSGILQPQQNCMEMPGPGHASAMSQDPSSRESDMLSSHQGQRSFSHVKDMKNEMLMHMMDGAQGSGSELIHDDAHTGSQLEFGVLNNHNSSSVPSMQSQGLSLSLNTQIMAPSLPYWSIKPDMLTPQSYHDNLRGEDMRMKNLQSEASRAIRNSRYLKAAQELLDEVVSVWKSIKQKAQKEKVESGKADGKETDGGPKSEGVSSNPQESGANAAPELSTAEKQELQNKMAKLMAMLDEVDRKYKHYYHQMQTVVSSFDVVAGPGSAKPYTAVALQTISRHFRCLKDAINDQINVIRKKLGEEENSSGKEGKLTRLRYIDQQLRQQRAFQQYGMIPQNAWRPQRGLPENSVTILRAWLFEHFLHPYPKDSEKLMLARQTGLTRSQISNWFINARVRLWKPMIEDMYKEEIGDLEQDSNSSSDNAPRSKDKMASSEDKEDLKNSRARICETSQLSESRTSIGAMNVGGAPVGFQNEPNPDDSFMNLMLKDQRSNEVDGGLLLHNTVAQHSDENARFMAYHLAELGRYGNGNVSLTLGLQHSSSNLVPNAQPGFPGVNEDDIYNATAPLGVTVASSDYDSMNQMDQRQRFEHSPLLHDFVA

SEQ ID NO: 7 - DNA, 1020 bp, (Arabidopsis thaliana)
  misc_feature 1..1020: note = AtDD45
  source 1..1020: mol_type = genomic DNA
aaatgttcctcgctgacgtaagaagacattagtaatggttataatatatagctttctatgaatgtatggtgagaaaatgtctgttcactgattttgagtttggaataaaagcatttgcgtttggtttatcattgcgtttatacaaggacagagatccactgagctggaatagcttaaaaccattatcagaacaaaataaaccattttttgttaagaatcagagcatagtaaacaacagaaacaacctaagagaggtaacttgtccaagaagatagctaattatatctattttataaaagttatcatagtttgtaagtcacaaaagatgcaaataacagagaaactaggagacttgagaatatacattcttgtatatttgtattcgagattgtgaaaatttgaccataagtttaaattcttaaaaagatatatctgatctagatgatggttatagactgtaattttaccacatgtttaatgatggatagtgacacacatgacacatcgacaacactatagcatcttatttagattacaacatgaaatttttctgtaatacatgtctttgtacataatttaaaagtaattcctaagaaatatatttatacaaggagtttaaagaaaacatagcataaagttcaatgagtagtaaaaaccatatacagtatatagcataaagttcaatgagtttattacaaaagcattggttcactttctgtaacacgacgttaaaccttcgtctccaataggagcgctactgattcaacatgccaatatatactaaatacgtttctacagtcaaatgctttaacgtttcatgattaagtgactatttaccgtcaatcctttcccattcctcccactaatccaactttttaattactcttaaatcaccactaagcttcgaatccatccaaaaccacaatataaaaacagaactctcgtaactcaatcatcgcaaaacaaaacaaaacaaaacaaaaaccccaaaaagaaagaataatggcttctaacacaagt